European Patent Application EP 4 394 033 A1, published July 3, 2024. Title: T CELL PRODUCT AND USE THEREOF. Applicant: Cells & Genes Biotech (Shanghai) Co.,Ltd. The sequence listing filed with the application follows.

SEQUENCE LISTING (12 sequences)

SEQ ID NO: 1 - DNA, 20 bp, synthetic construct
  misc_feature 1..20: note = sgRNA sequence targeting human CD3 gene
  source 1..20: mol_type = other DNA
tcagggttctggatatctgt

SEQ ID NO: 2 - DNA, 1461 bp, synthetic construct
  misc_feature 1..1461: note = nucleic acid encoding GPC3 CAR
  source 1..1461: mol_type = other DNA
atggccttaccagtgaccgccttgctcctgccgctggccttgctgctccacgccgccaggccgcaggtgcagctggtgcagtctggagctgaggtgaagaagcctggggcctcagtgaaggtctcctgcaaggcttctggatacaccttcaccgactatgaaatgcactgggtgcgacaggcccctggacaagggcttgagtggatgggagctcttgatcctaaaactggtgatactgcctacagtcagaagttcaagggcagagtcacgctgaccgcggacaaatccacgagcacagcctacatggagctgagcagcctgacatctgaggacacggccgtgtattactgtacaagattctactcctatacttactggggccagggaaccctggtcaccgtctcctcaggaggaggaggctctggaggaggagggagtggaggcgggggaagcgacgtggtgatgacccagagccccctgagcctgcccgtgacccccggcgagcccgccagcatcagctgcaggagcagccagagcctggtgcacagcaacggcaacacctacctgcactggtacctgcagaagcccggccagagcccccagctgctgatctacaaggtgagcaacaggttcagcggcgtgcccgacaggttcagcggcagcggcagcggcaccgacttcaccctgaagatcagcagggtggaggccgaggacgtgggcgtgtactactgcagccagaacacccacgtgccccccaccttcggccagggcaccaagctggagatcaagaccacgacgccagcgccgcgaccaccaacaccggcgcccaccatcgcgtcgcagcccctgtccctgcgcccagaggcgtgccggccagcggcggggggcgcagtgcacacgagggggctggacttcgcctgtgatatctacatctgggcgcccttggccgggacttgtggggtccttctcctgtcactggttatcaccctttactgcaaacggggcagaaagaaactcctgtatatattcaaacaaccatttatgagaccagtacaaactactcaagaggaagatggctgtagctgccgatttccagaagaagaagaaggaggatgtgaactgagagtgaagttcagcaggagcgcagacgcccccgcgtaccagcagggccagaaccagctctataacgagctcaatctaggacgaagagaggagtacgatgttttggacaagagacgtggccgggaccctgagatggggggaaagccgagaaggaagaaccctcaggaaggcctgtacaatgaactgcagaaagataagatggcggaggcctacagtgagattgggatgaaaggcgagcgccggaggggcaaggggcacgatggcctttaccagggtctcagtacagccaccaaggacacctacgacgcccttcacatgcaggccctgccccctcgctaa

SEQ ID NO: 3 - DNA, 1578 bp, synthetic construct
  misc_feature 1..1578: note = nucleic acid encoding GPC3 BITE
  source 1..1578: mol_type = other DNA
gccaccatgggatggagctgtatcatcctcttcttggtagcaacagctacaggtgtccactccgactacaaagatgatgacgataaggacgtggtgatgacccagagccccctgagcctgcccgtgacccccggcgagcccgccagcatcagctgcaggagcagccagagcctggtgcacagcaacggcaacacctacctgcactggtacctgcagaagcccggccagagcccccagctgctgatctacaaggtgagcaacaggttcagcggcgtgcccgacaggttcagcggcagcggcagcggcaccgacttcaccctgaagatcagcagggtggaggccgaggacgtgggcgtgtactactgcagccagaacacccacgtgccccccaccttcggccagggcaccaagctggagatcaagggaggaggaggctctggaggaggagggagtggaggcgggggaagccaggtgcagctggtgcagtctggagctgaggtgaagaagcctggggcctcagtgaaggtctcctgcaaggcttctggatacaccttcaccgactatgaaatgcactgggtgcgacaggcccctggacaagggcttgagtggatgggagctcttgatcctaaaactggtgatactgcctacagtcagaagttcaagggcagagtcacgctgaccgcggacaaatccacgagcacagcctacatggagctgagcagcctgacatctgaggacacggccgtgtattactgtacaagattctactcctatacttactggggccagggaaccctggtcaccgtctcctcaggaggtggtggatccgatatcaaactgcagcagtcaggggctgaactggcaagacctggggcctcagtgaagatgtcctgcaagacttctggctacacctttactaggtacacgatgcactgggtaaaacagaggcctggacagggtctggaatggattggatacattaatcctagccgtggttatactaattacaatcagaagttcaaggacaaggccacattgactacagacaaatcctccagcacagcctacatgcaactgagcagcctgacatctgaggactctgcagtctattactgtgcaagatattatgatgatcattactgccttgactactggggccaaggcaccactctcacagtctcctcagtcgaaggtggaagtggaggttctggtggaagtggaggttcaggtggagtcgacgacattcagctgacccagtctccagcaatcatgtctgcatctccaggggagaaggtcaccatgacctgcagagccagttcaagtgtaagttacatgaactggtaccagcagaagtcaggcacctcccccaaaagatggatttatgacacatccaaagtggcttctggagtcccttatcgcttcagtggcagtgggtctgggacctcatactctctcacaatcagcagcatggaggctgaagatgctgccacttattactgccaacagtggagtagtaacccgctcacgttcggtgctgggaccaagctggagctgaaacatcatcaccatcatcattag

SEQ ID NO: 4 - DNA, 4279 bp, synthetic construct
  misc_feature 1..4279: note = nucleic acid encoding GPC3 CAR BITE
  source 1..4279: mol_type = other DNA
cagtttgctttgctgggcctttttcccatgcctgcctttactctgccagagttatattgctggggttttgaagaagatcctattaaataaaagaataagcagtattattaagtagccctgcatttcaggtttccttgagtggcaggccaggcctggccgtgaacgttcactgaaatcatggcctcttggccaagattgatagcttgtgcctgtccctgagtcccagtccatcacgagcagctggtttctaagatgctatttcccgtataaagcatgagaccgtgacttgccagccccacagagccccgcccttgtccatcactggcatctggactccagcctgggttggggcaaagagggaaatgagatcatgtcctaaccctgatcctcttgtcccacactgacctcttctcttcctcccacagggcctcgagagatctggcagcggagagggcagaggaagtcttctaacatgcggtgacgtggaggagaatcccggccctaggctcgagatggccttaccagtgaccgccttgctcctgccgctggccttgctgctccacgccgccaggccgcaggtgcagctggtgcagtctggagctgaggtgaagaagcctggggcctcagtgaaggtctcctgcaaggcttctggatacaccttcaccgactatgaaatgcactgggtgcgacaggcccctggacaagggcttgagtggatgggagctcttgatcctaaaactggtgatactgcctacagtcagaagttcaagggcagagtcacgctgaccgcggacaaatccacgagcacagcctacatggagctgagcagcctgacatctgaggacacggccgtgtattactgtacaagattctactcctatacttactggggccagggaaccctggtcaccgtctcctcaggaggaggaggctctggaggaggagggagtggaggcgggggaagcgacgtggtgatgacccagagccccctgagcctgcccgtgacccccggcgagcccgccagcatcagctgcaggagcagccagagcctggtgcacagcaacggcaacacctacctgcactggtacctgcagaagcccggccagagcccccagctgctgatctacaaggtgagcaacaggttcagcggcgtgcccgacaggttcagcggcagcggcagcggcaccgacttcaccctgaagatcagcagggtggaggccgaggacgtgggcgtgtactactgcagccagaacacccacgtgccccccaccttcggccagggcaccaagctggagatcaagaccacgacgccagcgccgcgaccaccaacaccggcgcccaccatcgcgtcgcagcccctgtccctgcgcccagaggcgtgccggccagcggcggggggcgcagtgcacacgagggggctggacttcgcctgtgatatctacatctgggcgcccttggccgggacttgtggggtccttctcctgtcactggttatcaccctttactgcaaacggggcagaaagaaactcctgtatatattcaaacaaccatttatgagaccagtacaaactactcaagaggaagatggctgtagctgccgatttccagaagaagaagaaggaggatgtgaactgagagtgaagttcagcaggagcgcagacgcccccgcgtaccagcagggccagaaccagctctataacgagctcaatctaggacgaagagaggagtacgatgttttggacaagagacgtggccgggaccctgagatggggggaaagccgagaaggaagaaccctcaggaaggcctgtacaatgaactgcagaaagataagatggcggaggcctacagtgagattgggatgaaaggcgagcgccggaggggcaaggggcacgatggcctttaccagggtctcagtacagccaccaaggacacctacgacgcccttcacatgcaggccctgccccctcgcggcagcggcgccacaaacttctctctgctaaagcaagcaggtgatgttgaagaaaaccccgggcctatgggatggagctgtatcatcctcttcttggtagcaacagctacaggtgtccactccgactacaaagatgatgacgataaggacgtggtgatgacccagagccccctgagcctgcccgtgacccccggcgagcccgccagcatcagctgcaggagcagccagagcctggtgcacagcaacggcaacacctacctgcactggtacctgcagaagcccggccagagcccccagctgctgatctacaaggtgagcaacaggttcagcggcgtgcccgacaggttcagcggcagcggcagcggcaccgacttcaccctgaagatcagcagggtggaggccgaggacgtgggcgtgtactactgcagccagaacacccacgtgccccccaccttcggccagggcaccaagctggagatcaagggaggaggaggctctggaggaggagggagtggaggcgggggaagccaggtgcagctggtgcagtctggagctgaggtgaagaagcctggggcctcagtgaaggtctcctgcaaggcttctggatacaccttcaccgactatgaaatgcactgggtgcgacaggcccctggacaagggcttgagtggatgggagctcttgatcctaaaactggtgatactgcctacagtcagaagttcaagggcagagtcacgctgaccgcggacaaatccacgagcacagcctacatggagctgagcagcctgacatctgaggacacggccgtgtattactgtacaagattctactcctatacttactggggccagggaaccctggtcaccgtctcctcaggaggtggtggatccgatatcaaactgcagcagtcaggggctgaactggcaagacctggggcctcagtgaagatgtcctgcaagacttctggctacacctttactaggtacacgatgcactgggtaaaacagaggcctggacagggtctggaatggattggatacattaatcctagccgtggttatactaattacaatcagaagttcaaggacaaggccacattgactacagacaaatcctccagcacagcctacatgcaactgagcagcctgacatctgaggactctgcagtctattactgtgcaagatattatgatgatcattactgccttgactactggggccaaggcaccactctcacagtctcctcagtcgaaggtggaagtggaggttctggtggaagtggaggttcaggtggagtcgacgacattcagctgacccagtctccagcaatcatgtctgcatctccaggggagaaggtcaccatgacctgcagagccagttcaagtgtaagttacatgaactggtaccagcagaagtcaggcacctcccccaaaagatggatttatgacacatccaaagtggcttctggagtcccttatcgcttcagtggcagtgggtctgggacctcatactctctcacaatcagcagcatggaggctgaagatgctgccacttattactgccaacagtggagtagtaacccgctcacgttcggtgctgggaccaagctggagctgaaacatcatcaccatcatcattagctgtgccttctagttgccagccatctgttgtttgcccctcccccgtgccttccttgaccctggaaggtgccactcccactgtcctttcctaataaaatgaggaaattgcatcgcattgtctgagtaggtgtcattctattctggggggtggggtggggcaggacagcaagggggaggattgggaagacaatagcaggcatgctggggatgcggtgggctctatgggaattctctagaaatattctcgaggtttaaacgtcgacgcggccgcgatatccagaaccctgaccctgccgtgtaccagctgagagactctaaatccagtgacaagtctgtctgcctattcaccgattttgattctcaaacaaatgtgtcacaaagtaaggattctgatgtgtatatcacagacaaaactgtgctagacatgaggtctatggacttcaagagcaacagtgctgtggcctggagcaacaaatctgactttgcatgtgcaaacgccttcaacaacagcattattccagaagacaccttcttccccagcccaggtaagggcagctttggtgccttcgcaggctgtttccttgcttcaggaatggccaggttctgcccagagctctggtcaatgatgtctaaaactcctctgattggtggtctcggccttatccattgcc

SEQ ID NO: 5 - DNA, 519 bp, synthetic construct
  misc_feature 1..519: note = nucleic acid encoding cytokine IL1b
  source 1..519: mol_type = other DNA
atgggatggagctgtatcatcctcttcttggtagcaacagctacaggtgtccactccgcacctgtacgatcactgaactgcacgctccgggactcacagcaaaaaagcttggtgatgtctggtccatatgaactgaaagctctccacctccagggacaggatatggagcaacaagtggtgttctccatgtcctttgtacaaggagaagaaagtaatgacaaaatacctgtggccttgggcctcaaggaaaagaatctgtacctgtcctgcgtgttgaaagatgataagcccactctacagctggagagtgtagatcccaaaaattacccaaagaagaagatggaaaagcgatttgtcttcaacaagatagaaatcaataacaagctggaatttgagtctgcccagttccccaactggtacatcagcacctctcaagcagaaaacatgcccgtcttcctgggagggaccaaaggcggccaggatataactgacttcaccatgcaatttgtgtcttcctaa

SEQ ID NO: 6 - DNA, 465 bp, synthetic construct
  misc_feature 1..465: note = nucleic acid encoding chemokines CCL5
  source 1..465: mol_type = other DNA
atgaaggtctccgcggcagccctcgctgtcatcctcattgctactgccctctgcgctcctgcatctgcctccccatattcctcggacaccacaccctgctgctttgcctacattgcccgcccactgccccgtgcccacatcaaggagtatttctacaccagtggcaagtgctccaacccagcagtcgtccacaggtcaaggatgccaaagagagagggacagcaagtctggcaggatttcctgtatgactcccggctgaacaagggcaagctttgtcacccgaaagaaccgccaagtgtgtgccaacccagagaagaaatgggttcgggagtacatcaactctttggagatgagctaggatggagagtccttgaacctgaacttacacaaatttgcctgtttctgcttgctcttgtcctagcttgggaggcttcccctcactatcctaccccacccgctccttga

SEQ ID NO: 7 - DNA, 297 bp, synthetic construct
  misc_feature 1..297: note = nucleic acid encoding chemokine CXCL10
  source 1..297: mol_type = other DNA
atgaatcaaactgccattctgatttgctgccttatctttctgactctaagtggcattcaaggagtacctctctctagaactgtacgctgtacctgcatcagcattagtaatcaacctgttaatccaaggtctttagaaaaacttgaaattattcctgcaagccaattttgtccacgtgttgagatcattgctacaatgaaaaagaagggtgagaagagatgtctgaatccagaatcgaaggccatcaagaatttactgaaagcagttagcaaggaaaggtctaaaagatctccttaa

SEQ ID NO: 8 - DNA, 762 bp, synthetic construct
  misc_feature 1..762: note = nucleic acid encoding cytokine IL12-A
  source 1..762: mol_type = other DNA
atgtggccccctgggtcagcctcccagccaccgccctcacctgccgcggccacaggtctgcatccagcggctcgccctgtgtccctgcagtgccggctcagcatgtgtccagcgcgcagcctcctccttgtggctaccctggtcctcctggaccacctcagtttggccagaaacctccccgtggccactccagacccaggaatgttcccatgccttcaccactcccaaaacctgctgagggccgtcagcaacatgctccagaaggccagacaaactctagaattttacccttgcacttctgaagagattgatcatgaagatatcacaaaagataaaaccagcacagtggaggcctgtttaccattggaattaaccaagaatgagagttgcctaaattccagagagacctctttcataactaatgggagttgcctggcctccagaaagacctcttttatgatggccctgtgccttagtagtatttatgaagacttgaagatgtaccaggtggagttcaagaccatgaatgcaaagcttctgatggatcctaagaggcagatctttctagatcaaaacatgctggcagttattgatgagctgatgcaggccctgaatttcaacagtgagactgtgccacaaaaatcctcccttgaagaaccggatttttataaaactaaaatcaagctctgcatacttcttcatgctttcagaattcgggcagtgactattgatagagtgatgagctatctgaatgcttcctaa

SEQ ID NO: 9 - DNA, 987 bp, synthetic construct
  misc_feature 1..987: note = nucleic acid encoding cytokine IL12-B
  source 1..987: mol_type = other DNA
atgtgtcaccagcagttggtcatctcttggttttccctggtttttctggcatctcccctcgtggccatatgggaactgaagaaagatgtttatgtcgtagaattggattggtatccggatgcccctggagaaatggtggtcctcacctgtgacacccctgaagaagatggtatcacctggaccttggaccagagcagtgaggtcttaggctctggcaaaaccctgaccatccaagtcaaagagtttggagatgctggccagtacacctgtcacaaaggaggcgaggttctaagccattcgctcctgctgcttcacaaaaaggaagatggaatttggtccactgatattttaaaggaccagaaagaacccaaaaataagacctttctaagatgcgaggccaagaattattctggacgtttcacctgctggtggctgacgacaatcagtactgatttgacattcagtgtcaaaagcagcagaggctcttctgacccccaaggggtgacgtgcggagctgctacactctctgcagagagagtcagaggggacaacaaggagtatgagtactcagtggagtgccaggaggacagtgcctgcccagctgctgaggagagtctgcccattgaggtcatggtggatgccgttcacaagctcaagtatgaaaactacaccagcagcttcttcatcagggacatcatcaaacctgacccacccaagaacttgcagctgaagccattaaagaattctcggcaggtggaggtcagctgggagtaccctgacacctggagtactccacattcctacttctccctgacattctgcgttcaggtccagggcaagagcaagagagaaaagaaagatagagtcttcacggacaagacctcagccacggtcatctgccgcaaaaatgccagcattagcgtgcgggcccaggaccgctactatagctcatcttggagcgaatgggcatctgtgccctgcagttag

SEQ ID NO: 10 - protein, 857 aa, synthetic construct
  REGION 1..857: note = GPC3 CAR-2A-IL15-2A-IL-21
MALPVTALLLPLALLLHAARPQVQLVQSGAEVKKPGASVKVSCKASGYTFTDYEMHWVRQAPGQGLEWMGALDPKTGDTAYSQKFKGRVTLTADKSTSTAYMELSSLTSEDTAVYYCTRFYSYTYWGQGTLVTVSSGGGGSGGGGSGGGGSDVVMTQSPLSLPVTPGEPASISCRSSQSLVHSNGNTYLHWYLQKPGQSPQLLIYKVSNRFSGVPDRFSGSGSGTDFTLKISRVEAEDVGVYYCSQNTHVPPTFGQGTKLEIKTTTPAPRPPTPAPTIASQPLSLRPEACRPAAGGAVHTRGLDFACDIYIWAPLAGTCGVLLLSLVITLYCKRGRKKLLYIFKQPFMRPVQTTQEEDGCSCRFPEEEEGGCELRVKFSRSADAPAYQQGQNQLYNELNLGRREEYDVLDKRRGRDPEMGGKPRRKNPQEGLYNELQKDKMAEAYSEIGMKGERRRGKGHDGLYQGLSTATKDTYDALHMQALPPRGSGATNFSLLKQAGDVEENPGPMRISKPHLRSISIQCYLCLLLNSHFLTEAGIHVFILGCFSAGLPKTEANWVNVISDLKKIEDLIQSMHIDATLYTESDVHPSCKVTAMKCFLLELQVISLESGDASIHDTVENLIILANNSLSSNGNVTESGCKECEELEEKNIKEFLQSFVHIVQMFINTSGSGVKQTLNFDLLKLAGDVESNPGPMRSSPGNMERIVICLMVIFLGTLVHKSSSQGQDRHMIRMRQLIDIVDQLKNYVNDLVPEFLPAPEDVETNCEWSAFSCFQKAQLKSANTGNNERIINVSIKKLKRKPPSTNAGRRQKHRLTCPSCDSYEKKPPKEFLERFKSLLQKMIHQHLSSRTHGSEDS

SEQ ID NO: 11 - DNA, 2845 bp, synthetic construct
  misc_feature 1..2845: note = GPC3CAR-2A-IL15-2A-IL-21 (not include homologous arm)
  source 1..2845: mol_type = other DNA
atggccttaccagtgaccgccttgctcctgccgctggccttgctgctccacgccgccaggccgcaggtgcagctggtgcagtctggagctgaggtgaagaagcctggggcctcagtgaaggtctcctgcaaggcttctggatacaccttcaccgactatgaaatgcactgggtgcgacaggcccctggacaagggcttgagtggatgggagctcttgatcctaaaactggtgatactgcctacagtcagaagttcaagggcagagtcacgctgaccgcggacaaatccacgagcacagcctacatggagctgagcagcctgacatctgaggacacggccgtgtattactgtacaagattctactcctatacttactggggccagggaaccctggtcaccgtctcctcaggaggaggaggctctggaggaggagggagtggaggcgggggaagcgacgtggtgatgacccagagccccctgagcctgcccgtgacccccggcgagcccgccagcatcagctgcaggagcagccagagcctggtgcacagcaacggcaacacctacctgcactggtacctgcagaagcccggccagagcccccagctgctgatctacaaggtgagcaacaggttcagcggcgtgcccgacaggttcagcggcagcggcagcggcaccgacttcaccctgaagatcagcagggtggaggccgaggacgtgggcgtgtactactgcagccagaacacccacgtgccccccaccttcggccagggcaccaagctggagatcaagaccacgacgccagcgccgcgaccaccaacaccggcgcccaccatcgcgtcgcagcccctgtccctgcgcccagaggcgtgccggccagcggcggggggcgcagtgcacacgagggggctggacttcgcctgtgatatctacatctgggcgcccttggccgggacttgtggggtccttctcctgtcactggttatcaccctttactgcaaacggggcagaaagaaactcctgtatatattcaaacaaccatttatgagaccagtacaaactactcaagaggaagatggctgtagctgccgatttccagaagaagaagaaggaggatgtgaactgagagtgaagttcagcaggagcgcagacgcccccgcgtaccagcagggccagaaccagctctataacgagctcaatctaggacgaagagaggagtacgatgttttggacaagagacgtggccgggaccctgagatggggggaaagccgagaaggaagaaccctcaggaaggcctgtacaatgaactgcagaaagataagatggcggaggcctacagtgagattgggatgaaaggcgagcgccggaggggcaaggggcacgatggcctttaccagggtctcagtacagccaccaaggacacctacgacgcccttcacatgcaggccctgccccctcgcggcagcggcgccacaaacttctctctgctaaagcaagcaggtgatgttgaagaaaaccccgggcctatgagaatttcgaaaccacatttgagaagtatttccatccagtgctacttgtgtttacttctaaacagtcattttctaactgaagctggcattcatgtcttcattttgggctgtttcagtgcagggcttcctaaaacagaagccaactgggtgaatgtaataagtgatttgaaaaaaattgaagatcttattcaatctatgcatattgatgctactttatatacggaaagtgatgttcaccccagttgcaaagtaacagcaatgaagtgctttctcttggagttacaagttatttcacttgagtccggagatgcaagtattcatgatacagtagaaaatctgatcatcctagcaaacaacagtttgtcttctaatgggaatgtaacagaatctggatgcaaagaatgtgaggaactggaggaaaaaaatattaaagaatttttgcagagttttgtacatattgtccaaatgttcatcaacacttctggttctggcgtgaaacagactttgaattttgaccttctcaagttggcgggagacgtggagtccaacccagggcccatgagatccagtcctggcaacatggagaggattgtcatctgtctgatggtcatcttcttggggacactggtccacaaatcaagctcccaaggtcaagatcgccacatgattagaatgcgtcaacttatagatattgttgatcagctgaaaaattatgtgaatgacttggtccctgaatttctgccagctccagaagatgtagagacaaactgtgagtggtcagctttttcctgctttcagaaggcccaactaaagtcagcaaatacaggaaacaatgaaaggataatcaatgtatcaattaaaaagctgaagaggaaaccaccttccacaaatgcagggagaagacagaaacacagactaacatgcccttcatgtgattcttatgagaaaaaaccacccaaagaattcctagaaagattcaaatcacttctccaaaagatgattcatcagcatctgtcctctagaacacacggaagtgaagattcctgactgtgccttctagttgccagccatctgttgtttgcccctcccccgtgccttccttgaccctggaaggtgccactcccactgtcctttcctaataaaatgaggaaattgcatcgcattgtctgagtaggtgtcattctattctggggggtggggtggggcaggacagcaagggggaggattgggaagacaatagcaggcatgctggggatgcggtgggctctatgggaattctctagaaatattctcgaggtttaaacgtcgacgcggccgc

SEQ ID NO: 12 - DNA, 3757 bp, synthetic construct
  misc_feature 1..3757: note = GPC3CAR-2A-IL15-2A-IL-21 (include homologous arm)
  source 1..3757: mol_type = other DNA
cagtttgctttgctgggcctttttcccatgcctgcctttactctgccagagttatattgctggggttttgaagaagatcctattaaataaaagaataagcagtattattaagtagccctgcatttcaggtttccttgagtggcaggccaggcctggccgtgaacgttcactgaaatcatggcctcttggccaagattgatagcttgtgcctgtccctgagtcccagtccatcacgagcagctggtttctaagatgctatttcccgtataaagcatgagaccgtgacttgccagccccacagagccccgcccttgtccatcactggcatctggactccagcctgggttggggcaaagagggaaatgagatcatgtcctaaccctgatcctcttgtcccacactgacctcttctcttcctcccacagggcctcgagagatctggcagcggagagggcagaggaagtcttctaacatgcggtgacgtggaggagaatcccggccctaggctcgagatggccttaccagtgaccgccttgctcctgccgctggccttgctgctccacgccgccaggccgcaggtgcagctggtgcagtctggagctgaggtgaagaagcctggggcctcagtgaaggtctcctgcaaggcttctggatacaccttcaccgactatgaaatgcactgggtgcgacaggcccctggacaagggcttgagtggatgggagctcttgatcctaaaactggtgatactgcctacagtcagaagttcaagggcagagtcacgctgaccgcggacaaatccacgagcacagcctacatggagctgagcagcctgacatctgaggacacggccgtgtattactgtacaagattctactcctatacttactggggccagggaaccctggtcaccgtctcctcaggaggaggaggctctggaggaggagggagtggaggcgggggaagcgacgtggtgatgacccagagccccctgagcctgcccgtgacccccggcgagcccgccagcatcagctgcaggagcagccagagcctggtgcacagcaacggcaacacctacctgcactggtacctgcagaagcccggccagagcccccagctgctgatctacaaggtgagcaacaggttcagcggcgtgcccgacaggttcagcggcagcggcagcggcaccgacttcaccctgaagatcagcagggtggaggccgaggacgtgggcgtgtactactgcagccagaacacccacgtgccccccaccttcggccagggcaccaagctggagatcaagaccacgacgccagcgccgcgaccaccaacaccggcgcccaccatcgcgtcgcagcccctgtccctgcgcccagaggcgtgccggccagcggcggggggcgcagtgcacacgagggggctggacttcgcctgtgatatctacatctgggcgcccttggccgggacttgtggggtccttctcctgtcactggttatcaccctttactgcaaacggggcagaaagaaactcctgtatatattcaaacaaccatttatgagaccagtacaaactactcaagaggaagatggctgtagctgccgatttccagaagaagaagaaggaggatgtgaactgagagtgaagttcagcaggagcgcagacgcccccgcgtaccagcagggccagaaccagctctataacgagctcaatctaggacgaagagaggagtacgatgttttggacaagagacgtggccgggaccctgagatggggggaaagccgagaaggaagaaccctcaggaaggcctgtacaatgaactgcagaaagataagatggcggaggcctacagtgagattgggatgaaaggcgagcgccggaggggcaaggggcacgatggcctttaccagggtctcagtacagccaccaaggacacctacgacgcccttcacatgcaggccctgccccctcgcggcagcggcgccacaaacttctctctgctaaagcaagcaggtgatgttgaagaaaaccccgggcctatgagaatttcgaaaccacatttgagaagtatttccatccagtgctacttgtgtttacttctaaacagtcattttctaactgaagctggcattcatgtcttcattttgggctgtttcagtgcagggcttcctaaaacagaagccaactgggtgaatgtaataagtgatttgaaaaaaattgaagatcttattcaatctatgcatattgatgctactttatatacggaaagtgatgttcaccccagttgcaaagtaacagcaatgaagtgctttctcttggagttacaagttatttcacttgagtccggagatgcaagtattcatgatacagtagaaaatctgatcatcctagcaaacaacagtttgtcttctaatgggaatgtaacagaatctggatgcaaagaatgtgaggaactggaggaaaaaaatattaaagaatttttgcagagttttgtacatattgtccaaatgttcatcaacacttctggttctggcgtgaaacagactttgaattttgaccttctcaagttggcgggagacgtggagtccaacccagggcccatgagatccagtcctggcaacatggagaggattgtcatctgtctgatggtcatcttcttggggacactggtccacaaatcaagctcccaaggtcaagatcgccacatgattagaatgcgtcaacttatagatattgttgatcagctgaaaaattatgtgaatgacttggtccctgaatttctgccagctccagaagatgtagagacaaactgtgagtggtcagctttttcctgctttcagaaggcccaactaaagtcagcaaatacaggaaacaatgaaaggataatcaatgtatcaattaaaaagctgaagaggaaaccaccttccacaaatgcagggagaagacagaaacacagactaacatgcccttcatgtgattcttatgagaaaaaaccacccaaagaattcctagaaagattcaaatcacttctccaaaagatgattcatcagcatctgtcctctagaacacacggaagtgaagattcctgactgtgccttctagttgccagccatctgttgtttgcccctcccccgtgccttccttgaccctggaaggtgccactcccactgtcctttcctaataaaatgaggaaattgcatcgcattgtctgagtaggtgtcattctattctggggggtggggtggggcaggacagcaagggggaggattgggaagacaatagcaggcatgctggggatgcggtgggctctatgggaattctctagaaatattctcgaggtttaaacgtcgacgcggccgcgatatccagaaccctgaccctgccgtgtaccagctgagagactctaaatccagtgacaagtctgtctgcctattcaccgattttgattctcaaacaaatgtgtcacaaagtaaggattctgatgtgtatatcacagacaaaactgtgctagacatgaggtctatggacttcaagagcaacagtgctgtggcctggagcaacaaatctgactttgcatgtgcaaacgccttcaacaacagcattattccagaagacaccttcttccccagcccaggtaagggcagctttggtgccttcgcaggctgtttccttgcttcaggaatggccaggttctgcccagagctctggtcaatgatgtctaaaactcctctgattggtggtctcggccttatccattgcc